European Patent Application EP 4 177 352 A1, published May 10, 2023. Title: A microsphere comprising a first material and a second material. Applicant: BLINK AG. The sequence listing filed with the application follows.

SEQUENCE LISTING (9 sequences)

SEQ ID NO: 1 - DNA, 24 bp, Artificial Sequence
  "sense primer for mecA"
  sense primer for mecA
tggcatgagtaacgaagaatataa

SEQ ID NO: 2 - DNA, 21 bp, Artificial Sequence
  "antisense primer for mecA"
  antisense primer for mecA
gagttgaacctggtgaagttg

SEQ ID NO: 3 - DNA, 28 bp, Artificial Sequence
  "TaqMan probe for mecA"
  TaqMan probe for mecA
  misc_feature 1: /note="Atto647N-label"
  misc_feature 28: /note="BHQ2 label"
aaagaacctctgctcaacaagttccaga

SEQ ID NO: 4 - DNA, 20 bp, Artificial Sequence
  "sense primer for HCV"
  sense primer for HCV
gtggtctgcggaaccggtga

SEQ ID NO: 5 - DNA, 22 bp, Artificial Sequence
  "antisense primer for HCV"
  antisense primer for HCV
cgcaagcaccctatcaggcagt

SEQ ID NO: 6 - DNA, 25 bp, Artificial Sequence
  "TaqMan probe for HCV"
  TaqMan probe for HCV
  misc_feature 1: /note="Atto488-label"
  misc_feature 25: /note="BHQ1-label"
ccgagtagcgttgggttgcgaaagg

SEQ ID NO: 7 - DNA, 22 bp, Artificial Sequence
  "forward primer for gapA of Staphylococcus aureus"
  forward primer for gapA of Staphylococcus aureus
  misc_feature 1: /note="desthiobiotin-tag"
cgtcaattagttaaagttgcag

SEQ ID NO: 8 - DNA, 23 bp, Artificial Sequence
  "reverse primer for gapA of Staphylococcus aureus"
  reverse primer for gapA of Staphylococcus aureus
  misc_feature 1: /note="desthiobiotin-tag"
gctaagtatgctaatgtacgaac

SEQ ID NO: 9 - DNA, 31 bp, Artificial Sequence
  "probe for gapA of Staphylococcus aureus"
  probe for gapA of Staphylococcus aureus
  misc_feature 1: /note="desthiobiotin"
  misc_feature 31: /note="Cy5-label"
tggtatgataacgaaatgtcatatactgcac